European Patent Application EP 4 424 834 A2, published September 4, 2024. Title: MICROORGANISM HAVING INCREASED ACTIVITY OF 3-METHYL-2-OXOBUTANOATE HYDROXYMETHYLTRANSFERASE, AND USE THEREOF. Applicant: CJ CheilJedang Corporation. The sequence listing filed with the application follows.

SEQUENCE LISTING (73 sequences)

SEQ ID NO: 1 - DNA, 37 bp, synthetic construct
  misc_feature 1..37: note = synthetic_primer
  source 1..37: mol_type = other DNA
tagatcgaaaggtgcacaaagatgaaaccgaccacca

SEQ ID NO: 2 - DNA, 41 bp, synthetic construct
  misc_feature 1..41: note = synthetic_primer
  source 1..41: mol_type = other DNA
ccgctctagaactagtggatcttaatggaaactgtgttctt

SEQ ID NO: 3 - DNA, 36 bp, synthetic construct
  misc_feature 1..36: note = synthetic_primer
  source 1..36: mol_type = other DNA
tagatcgaaaggtgcacaaagatgaaaccgaccacc

SEQ ID NO: 4 - DNA, 40 bp, synthetic construct
  misc_feature 1..40: note = synthetic_primer
  source 1..40: mol_type = other DNA
ccgctctagaactagtggatcttaatggaaactgtgttct

SEQ ID NO: 5 - DNA, 38 bp, synthetic construct
  misc_feature 1..38: note = synthetic_primer
  source 1..38: mol_type = other DNA
tagatcgaaaggtgcacaaagatgaaaccaaccaccat

SEQ ID NO: 6 - DNA, 41 bp, synthetic construct; identical to SEQ ID NO: 2
  misc_feature 1..41: note = synthetic_primer
  source 1..41: mol_type = other DNA

SEQ ID NO: 7 - DNA, 42 bp, synthetic construct
  misc_feature 1..42: note = synthetic_primer
  source 1..42: mol_type = other DNA
tagatcgaaaggtgcacaaagatgtcattaaagcaaataact

SEQ ID NO: 8 - DNA, 41 bp, synthetic construct
  misc_feature 1..41: note = synthetic_primer
  source 1..41: mol_type = other DNA
ccgctctagaactagtggatcttattggaaactgtgttctt

SEQ ID NO: 9 - DNA, 36 bp, synthetic construct
  misc_feature 1..36: note = synthetic_primer
  source 1..36: mol_type = other DNA
tagatcgaaaggtgcacaaagatgaaacccaccacc

SEQ ID NO: 10 - DNA, 39 bp, synthetic construct
  misc_feature 1..39: note = synthetic_primer
  source 1..39: mol_type = other DNA
ccgctctagaactagtggatcttagttaaatgagtgctc

SEQ ID NO: 11 - DNA, 37 bp, synthetic construct; identical to SEQ ID NO: 1
  misc_feature 1..37: note = synthetic_primer
  source 1..37: mol_type = other DNA

SEQ ID NO: 12 - DNA, 40 bp, synthetic construct; identical to SEQ ID NO: 4
  misc_feature 1..40: note = synthetic_primer
  source 1..40: mol_type = other DNA

SEQ ID NO: 13 - DNA, 36 bp, synthetic construct
  misc_feature 1..36: note = synthetic_primer
  source 1..36: mol_type = other DNA
tagatcgaaaggtgcacaaagatgaaacccaccacg

SEQ ID NO: 14 - DNA, 38 bp, synthetic construct
  misc_feature 1..38: note = synthetic_primer
  source 1..38: mol_type = other DNA
ccgctctagaactagtggatcttactggaaactgtgct

SEQ ID NO: 15 - DNA, 44 bp, synthetic construct
  misc_feature 1..44: note = synthetic_primer
  source 1..44: mol_type = other DNA
tagatcgaaaggtgcacaaagatgaaaactttaaatcatttaaa

SEQ ID NO: 16 - DNA, 39 bp, synthetic construct
  misc_feature 1..39: note = synthetic_primer
  source 1..39: mol_type = other DNA
ccgctctagaactagtggatcttagtcatgttgctctac

SEQ ID NO: 17 - DNA, 37 bp, synthetic construct
  misc_feature 1..37: note = synthetic_primer
  source 1..37: mol_type = other DNA
tagatcgaaaggtgcacaaagatgccagatgtaaccg

SEQ ID NO: 18 - DNA, 36 bp, synthetic construct
  misc_feature 1..36: note = synthetic_primer
  source 1..36: mol_type = other DNA
ccgctctagaactagtggatctcatgcggagaaccc

SEQ ID NO: 19 - DNA, 36 bp, synthetic construct
  misc_feature 1..36: note = synthetic_primer
  source 1..36: mol_type = other DNA
tagatcgaaaggtgcacaaagatgcctgatgtgacc

SEQ ID NO: 20 - DNA, 36 bp, synthetic construct
  misc_feature 1..36: note = synthetic_primer
  source 1..36: mol_type = other DNA
ccgctctagaactagtggatctcatgcggagaatcc

SEQ ID NO: 21 - DNA, 39 bp, synthetic construct
  misc_feature 1..39: note = synthetic_primer
  source 1..39: mol_type = other DNA
tagatcgaaaggtgcacaaagatgtcggtacataaagaa

SEQ ID NO: 22 - DNA, 42 bp, synthetic construct
  misc_feature 1..42: note = synthetic_primer
  source 1..42: mol_type = other DNA
ccgctctagaactagtggatcttaatattgttctttttcgtt

SEQ ID NO: 23 - DNA, 36 bp, synthetic construct; identical to SEQ ID NO: 9
  misc_feature 1..36: note = synthetic_primer
  source 1..36: mol_type = other DNA

SEQ ID NO: 24 - DNA, 40 bp, synthetic construct
  misc_feature 1..40: note = synthetic_primer
  source 1..40: mol_type = other DNA
ccgctctagaactagtggatcttagttgaaagagtgctct

SEQ ID NO: 25 - DNA, 40 bp, synthetic construct
  misc_feature 1..40: note = synthetic_primer
  source 1..40: mol_type = other DNA
tagatcgaaaggtgcacaaagatgtctacagcaaaaaaag

SEQ ID NO: 26 - DNA, 40 bp, synthetic construct
  misc_feature 1..40: note = synthetic_primer
  source 1..40: mol_type = other DNA
ccgctctagaactagtggatcttaatactgttcatcgtca

SEQ ID NO: 27 - DNA, 41 bp, synthetic construct
  misc_feature 1..41: note = synthetic_primer
  source 1..41: mol_type = other DNA
cttgatatcgaattcctgcattcagggtagttgactaaaga

SEQ ID NO: 28 - DNA, 17 bp, synthetic construct
  misc_feature 1..17: note = synthetic_primer
  source 1..17: mol_type = other DNA
ctttgtgcacctttcga

SEQ ID NO: 29 - DNA, 40 bp, synthetic construct
  misc_feature 1..40: note = synthetic_primer
  source 1..40: mol_type = other DNA
tgaattcgagctcggtacccgaaatagcgcttgatgaatc

SEQ ID NO: 30 - DNA, 40 bp, synthetic construct
  misc_feature 1..40: note = synthetic_primer
  source 1..40: mol_type = other DNA
ggttgctacctgcacccggggggcatgagtatagatgtga

SEQ ID NO: 31 - DNA, 40 bp, synthetic construct
  misc_feature 1..40: note = synthetic_primer
  source 1..40: mol_type = other DNA
ctatactcatgccccccgggtgcaggtagcaaccacaaag

SEQ ID NO: 32 - DNA, 40 bp, synthetic construct
  misc_feature 1..40: note = synthetic_primer
  source 1..40: mol_type = other DNA
gtcgactctagaggatcccctatgtggcgttgggtgcagc

SEQ ID NO: 33 - DNA, 40 bp, synthetic construct
  misc_feature 1..40: note = synthetic_primer
  source 1..40: mol_type = other DNA
catctatactcatgccccccttcagggtagttgactaaag

SEQ ID NO: 34 - DNA, 40 bp, synthetic construct
  misc_feature 1..40: note = synthetic_primer
  source 1..40: mol_type = other DNA
tgtggttgctacctgcacccttaatggaaactgtgttctt

SEQ ID NO: 35 - DNA, 20 bp, synthetic construct
  misc_feature 1..20: note = synthetic_primer
  source 1..20: mol_type = other DNA
cccacccggtgtcattcgac

SEQ ID NO: 36 - DNA, 19 bp, synthetic construct
  misc_feature 1..19: note = synthetic_primer
  source 1..19: mol_type = other DNA
gcgcatccagctcatcggt

SEQ ID NO: 37 - protein, 264 aa, synthetic construct
  REGION 1..264: note = synthetic_PanB WT
MKPTTISLLQKYKQEKKRFATITAYDYSFAKLFADEGLNVMLVGDSLGMTVQGHDSTLPVTVADIAYHTAAVRRGAPNCLLLADLPFMAYATPEQAFENAATVMRAGANMVKIEGGEWLVETVQMLTERAVPVCGHLGLTPQSVNIFGGYKVQGRGDEAGDQLLSDALALEAAGAQLLVLECVPVELAKRITEALAIPVIGIGAGNVTDGQILVMHDAFGITGGHIPKFAKNFLAETGDIRAAVRQYMAEVESGVYPGEEHSFH

SEQ ID NO: 38 - DNA, 40 bp, synthetic construct
  misc_feature 1..40: note = synthetic_primer
  source 1..40: mol_type = other DNA
gtttctaccagccactcggagccttcaattttgaccatgt

SEQ ID NO: 39 - DNA, 40 bp, synthetic construct
  misc_feature 1..40: note = synthetic_primer
  source 1..40: mol_type = other DNA
acatggtcaaaattgaaggctccgagtggctggtagaaac

SEQ ID NO: 40 - DNA, 40 bp, synthetic construct
  misc_feature 1..40: note = synthetic_primer
  source 1..40: mol_type = other DNA
gtttctaccagccactcgcagccttcaattttgaccatgt

SEQ ID NO: 41 - DNA, 40 bp, synthetic construct
  misc_feature 1..40: note = synthetic_primer
  source 1..40: mol_type = other DNA
acatggtcaaaattgaaggctgcgagtggctggtagaaac

SEQ ID NO: 42 - DNA, 40 bp, synthetic construct
  misc_feature 1..40: note = synthetic_primer
  source 1..40: mol_type = other DNA
gtttctaccagccactccaggccttcaattttgaccatgt

SEQ ID NO: 43 - DNA, 40 bp, synthetic construct
  misc_feature 1..40: note = synthetic_primer
  source 1..40: mol_type = other DNA
acatggtcaaaattgaaggcctggagtggctggtagaaac

SEQ ID NO: 44 - DNA, 40 bp, synthetic construct
  misc_feature 1..40: note = synthetic_primer
  source 1..40: mol_type = other DNA
gtttctaccagccactcgatgccttcaattttgaccatgt

SEQ ID NO: 45 - DNA, 40 bp, synthetic construct
  misc_feature 1..40: note = synthetic_primer
  source 1..40: mol_type = other DNA
acatggtcaaaattgaaggcatcgagtggctggtagaaac

SEQ ID NO: 46 - DNA, 40 bp, synthetic construct
  misc_feature 1..40: note = synthetic_primer
  source 1..40: mol_type = other DNA
gtttctaccagccactcggtgccttcaattttgaccatgt

SEQ ID NO: 47 - DNA, 40 bp, synthetic construct
  misc_feature 1..40: note = synthetic_primer
  source 1..40: mol_type = other DNA
acatggtcaaaattgaaggcaccgagtggctggtagaaac

SEQ ID NO: 48 - DNA, 40 bp, synthetic construct
  misc_feature 1..40: note = synthetic_primer
  source 1..40: mol_type = other DNA
gtttctaccagccactccacgccttcaattttgaccatgt

SEQ ID NO: 49 - DNA, 40 bp, synthetic construct
  misc_feature 1..40: note = synthetic_primer
  source 1..40: mol_type = other DNA
acatggtcaaaattgaaggcgtggagtggctggtagaaac

SEQ ID NO: 50 - DNA, 40 bp, synthetic construct
  misc_feature 1..40: note = synthetic_primer
  source 1..40: mol_type = other DNA
gtttctaccagccactccatgccttcaattttgaccatgt

SEQ ID NO: 51 - DNA, 40 bp, synthetic construct
  misc_feature 1..40: note = synthetic_primer
  source 1..40: mol_type = other DNA
acatggtcaaaattgaaggcatggagtggctggtagaaac

SEQ ID NO: 52 - DNA, 40 bp, synthetic construct
  misc_feature 1..40: note = synthetic_primer
  source 1..40: mol_type = other DNA
gtttctaccagccactcatcgccttcaattttgaccatgt

SEQ ID NO: 53 - DNA, 40 bp, synthetic construct
  misc_feature 1..40: note = synthetic_primer
  source 1..40: mol_type = other DNA
acatggtcaaaattgaaggcgatgagtggctggtagaaac

SEQ ID NO: 54 - DNA, 40 bp, synthetic construct
  misc_feature 1..40: note = synthetic_primer
  source 1..40: mol_type = other DNA
gtttctaccagccactcttcgccttcaattttgaccatgt

SEQ ID NO: 55 - DNA, 40 bp, synthetic construct
  misc_feature 1..40: note = synthetic_primer
  source 1..40: mol_type = other DNA
acatggtcaaaattgaaggcgaagagtggctggtagaaac

SEQ ID NO: 56 - DNA, 40 bp, synthetic construct
  misc_feature 1..40: note = synthetic_primer
  source 1..40: mol_type = other DNA
gtttctaccagccactcgttgccttcaattttgaccatgt

SEQ ID NO: 57 - DNA, 40 bp, synthetic construct
  misc_feature 1..40: note = synthetic_primer
  source 1..40: mol_type = other DNA
acatggtcaaaattgaaggcaacgagtggctggtagaaac

SEQ ID NO: 58 - DNA, 40 bp, synthetic construct
  misc_feature 1..40: note = synthetic_primer
  source 1..40: mol_type = other DNA
gtttctaccagccactcctggccttcaattttgaccatgt

SEQ ID NO: 59 - DNA, 40 bp, synthetic construct
  misc_feature 1..40: note = synthetic_primer
  source 1..40: mol_type = other DNA
acatggtcaaaattgaaggccaggagtggctggtagaaac

SEQ ID NO: 60 - DNA, 40 bp, synthetic construct
  misc_feature 1..40: note = synthetic_primer
  source 1..40: mol_type = other DNA
gtttctaccagccactctgcgccttcaattttgaccatgt

SEQ ID NO: 61 - DNA, 40 bp, synthetic construct
  misc_feature 1..40: note = synthetic_primer
  source 1..40: mol_type = other DNA
acatggtcaaaattgaaggcgcagagtggctggtagaaac

SEQ ID NO: 62 - protein, 264 aa, synthetic construct
  REGION 1..264: note = synthetic_PanB with G116A mutation
MKPTTISLLQKYKQEKKRFATITAYDYSFAKLFADEGLNVMLVGDSLGMTVQGHDSTLPVTVADIAYHTAAVRRGAPNCLLLADLPFMAYATPEQAFENAATVMRAGANMVKIEGAEWLVETVQMLTERAVPVCGHLGLTPQSVNIFGGYKVQGRGDEAGDQLLSDALALEAAGAQLLVLECVPVELAKRITEALAIPVIGIGAGNVTDGQILVMHDAFGITGGHIPKFAKNFLAETGDIRAAVRQYMAEVESGVYPGEEHSFH

SEQ ID NO: 63 - protein, 264 aa, synthetic construct
  REGION 1..264: note = synthetic_PanB with G116N mutation
MKPTTISLLQKYKQEKKRFATITAYDYSFAKLFADEGLNVMLVGDSLGMTVQGHDSTLPVTVADIAYHTAAVRRGAPNCLLLADLPFMAYATPEQAFENAATVMRAGANMVKIEGNEWLVETVQMLTERAVPVCGHLGLTPQSVNIFGGYKVQGRGDEAGDQLLSDALALEAAGAQLLVLECVPVELAKRITEALAIPVIGIGAGNVTDGQILVMHDAFGITGGHIPKFAKNFLAETGDIRAAVRQYMAEVESGVYPGEEHSFH

SEQ ID NO: 64 - protein, 264 aa, synthetic construct
  REGION 1..264: note = synthetic_PanB with G116T mutation
MKPTTISLLQKYKQEKKRFATITAYDYSFAKLFADEGLNVMLVGDSLGMTVQGHDSTLPVTVADIAYHTAAVRRGAPNCLLLADLPFMAYATPEQAFENAATVMRAGANMVKIEGTEWLVETVQMLTERAVPVCGHLGLTPQSVNIFGGYKVQGRGDEAGDQLLSDALALEAAGAQLLVLECVPVELAKRITEALAIPVIGIGAGNVTDGQILVMHDAFGITGGHIPKFAKNFLAETGDIRAAVRQYMAEVESGVYPGEEHSFH

SEQ ID NO: 65 - protein, 264 aa, synthetic construct
  REGION 1..264: note = synthetic_PanB with G116E mutation
MKPTTISLLQKYKQEKKRFATITAYDYSFAKLFADEGLNVMLVGDSLGMTVQGHDSTLPVTVADIAYHTAAVRRGAPNCLLLADLPFMAYATPEQAFENAATVMRAGANMVKIEGEEWLVETVQMLTERAVPVCGHLGLTPQSVNIFGGYKVQGRGDEAGDQLLSDALALEAAGAQLLVLECVPVELAKRITEALAIPVIGIGAGNVTDGQILVMHDAFGITGGHIPKFAKNFLAETGDIRAAVRQYMAEVESGVYPGEEHSFH

SEQ ID NO: 66 - protein, 264 aa, synthetic construct
  REGION 1..264: note = synthetic_PanB with G116S mutation
MKPTTISLLQKYKQEKKRFATITAYDYSFAKLFADEGLNVMLVGDSLGMTVQGHDSTLPVTVADIAYHTAAVRRGAPNCLLLADLPFMAYATPEQAFENAATVMRAGANMVKIEGSEWLVETVQMLTERAVPVCGHLGLTPQSVNIFGGYKVQGRGDEAGDQLLSDALALEAAGAQLLVLECVPVELAKRITEALAIPVIGIGAGNVTDGQILVMHDAFGITGGHIPKFAKNFLAETGDIRAAVRQYMAEVESGVYPGEEHSFH

SEQ ID NO: 67 - protein, 264 aa, synthetic construct
  REGION 1..264: note = synthetic_PanB with G116V mutation
MKPTTISLLQKYKQEKKRFATITAYDYSFAKLFADEGLNVMLVGDSLGMTVQGHDSTLPVTVADIAYHTAAVRRGAPNCLLLADLPFMAYATPEQAFENAATVMRAGANMVKIEGVEWLVETVQMLTERAVPVCGHLGLTPQSVNIFGGYKVQGRGDEAGDQLLSDALALEAAGAQLLVLECVPVELAKRITEALAIPVIGIGAGNVTDGQILVMHDAFGITGGHIPKFAKNFLAETGDIRAAVRQYMAEVESGVYPGEEHSFH

SEQ ID NO: 68 - protein, 264 aa, synthetic construct
  REGION 1..264: note = synthetic_PanB with G116I mutation
MKPTTISLLQKYKQEKKRFATITAYDYSFAKLFADEGLNVMLVGDSLGMTVQGHDSTLPVTVADIAYHTAAVRRGAPNCLLLADLPFMAYATPEQAFENAATVMRAGANMVKIEGIEWLVETVQMLTERAVPVCGHLGLTPQSVNIFGGYKVQGRGDEAGDQLLSDALALEAAGAQLLVLECVPVELAKRITEALAIPVIGIGAGNVTDGQILVMHDAFGITGGHIPKFAKNFLAETGDIRAAVRQYMAEVESGVYPGEEHSFH

SEQ ID NO: 69 - protein, 264 aa, synthetic construct
  REGION 1..264: note = synthetic_PanB with G116L mutation
MKPTTISLLQKYKQEKKRFATITAYDYSFAKLFADEGLNVMLVGDSLGMTVQGHDSTLPVTVADIAYHTAAVRRGAPNCLLLADLPFMAYATPEQAFENAATVMRAGANMVKIEGLEWLVETVQMLTERAVPVCGHLGLTPQSVNIFGGYKVQGRGDEAGDQLLSDALALEAAGAQLLVLECVPVELAKRITEALAIPVIGIGAGNVTDGQILVMHDAFGITGGHIPKFAKNFLAETGDIRAAVRQYMAEVESGVYPGEEHSFH

SEQ ID NO: 70 - protein, 264 aa, synthetic construct
  REGION 1..264: note = synthetic_PanB with G116D mutation
MKPTTISLLQKYKQEKKRFATITAYDYSFAKLFADEGLNVMLVGDSLGMTVQGHDSTLPVTVADIAYHTAAVRRGAPNCLLLADLPFMAYATPEQAFENAATVMRAGANMVKIEGDEWLVETVQMLTERAVPVCGHLGLTPQSVNIFGGYKVQGRGDEAGDQLLSDALALEAAGAQLLVLECVPVELAKRITEALAIPVIGIGAGNVTDGQILVMHDAFGITGGHIPKFAKNFLAETGDIRAAVRQYMAEVESGVYPGEEHSFH

SEQ ID NO: 71 - protein, 264 aa, synthetic construct
  REGION 1..264: note = synthetic_PanB with G116C mutation
MKPTTISLLQKYKQEKKRFATITAYDYSFAKLFADEGLNVMLVGDSLGMTVQGHDSTLPVTVADIAYHTAAVRRGAPNCLLLADLPFMAYATPEQAFENAATVMRAGANMVKIEGCEWLVETVQMLTERAVPVCGHLGLTPQSVNIFGGYKVQGRGDEAGDQLLSDALALEAAGAQLLVLECVPVELAKRITEALAIPVIGIGAGNVTDGQILVMHDAFGITGGHIPKFAKNFLAETGDIRAAVRQYMAEVESGVYPGEEHSFH

SEQ ID NO: 72 - protein, 264 aa, synthetic construct
  REGION 1..264: note = synthetic_PanB with G116Q mutation
MKPTTISLLQKYKQEKKRFATITAYDYSFAKLFADEGLNVMLVGDSLGMTVQGHDSTLPVTVADIAYHTAAVRRGAPNCLLLADLPFMAYATPEQAFENAATVMRAGANMVKIEGQEWLVETVQMLTERAVPVCGHLGLTPQSVNIFGGYKVQGRGDEAGDQLLSDALALEAAGAQLLVLECVPVELAKRITEALAIPVIGIGAGNVTDGQILVMHDAFGITGGHIPKFAKNFLAETGDIRAAVRQYMAEVESGVYPGEEHSFH

SEQ ID NO: 73 - protein, 264 aa, synthetic construct
  REGION 1..264: note = synthetic_PanB with G116M mutation
MKPTTISLLQKYKQEKKRFATITAYDYSFAKLFADEGLNVMLVGDSLGMTVQGHDSTLPVTVADIAYHTAAVRRGAPNCLLLADLPFMAYATPEQAFENAATVMRAGANMVKIEGMEWLVETVQMLTERAVPVCGHLGLTPQSVNIFGGYKVQGRGDEAGDQLLSDALALEAAGAQLLVLECVPVELAKRITEALAIPVIGIGAGNVTDGQILVMHDAFGITGGHIPKFAKNFLAETGDIRAAVRQYMAEVESGVYPGEEHSFH